European Patent Specification EP 3 700 915 B1, published June 18, 2025. Title: BACTERIAL LEADER SEQUENCES FOR PERIPLASMIC PROTEIN EXPRESSION. Applicant: PFENEX INC. The sequence listing filed with the application follows.

SEQUENCE LISTING (20 sequences)

SEQ ID NO: 1 - protein, 25 aa, Pseudomonas fluorescens
MKSALKNVIPGALALLLLFPVAAQA

SEQ ID NO: 2 - protein, 18 aa, Pseudomonas fluorescens
MRQLFFCLMLMVSLTAHA

SEQ ID NO: 3 - protein, 29 aa, Pseudomonas fluorescens
MQSLPFSALRLLGVLAVMVCVLLTTPARA

SEQ ID NO: 4 - DNA, 75 bp, Pseudomonas fluorescens
atgaaatctgcattgaagaacgttattccgggcgccctggcccttctgctgctattccccgtcgccgcccaggcc

SEQ ID NO: 5 - DNA, 54 bp, Pseudomonas fluorescens
atgcgacaactatttttctgtttgatgctgatggtgtcgctcacggcgcacgcc

SEQ ID NO: 6 - DNA, 87 bp, Pseudomonas fluorescens
atgcaaagcctgccgttctctgcgttacgcctgctcggtgtgctggcagtcatggtctgcgtgctgttgacgacgccagcccgtgcc

SEQ ID NO: 7 - protein, 327 aa, Erwinia chrysanthemi
ADKLPNIVILATGGTIAGSAATGTQTTGYKAGALGVDTLINAVPEVKKLANVKGEQFSNMASENMTGDVVLKLSQRVNELLARDDVDGVVITHGTDTVEESAYFLHLTVKSDKPVVFVAAMRPATAISADGPMNLLEAVRVAGDKQSRGRGVMVVLNDRIGSARYITKTNASTLDTFKANEEGYLGVIIGNRIYYQNRIDKLHTTRSVFDVRGLTSLPKVDILYGYQDDPEYLYDAAIQHGVKGIVYAGMGAGSVSVRGIAGMRKAMEKGVVVIRSTRTGNGIVPPDEELPGLVSDSLNPAHARILLMLALTRTSDPKVIQEYFHTY

SEQ ID NO: 8 - DNA, 981 bp, Artificial Sequence
  Description of Artificial Sequence: Synthetic polynucleotide
gcagacaaactccctaacatcgtaatcctcgcaactggtggtaccatcgcaggcagcgccgccaccggcacgcagaccactggctacaaggccggcgcgctgggcgtagacacgctgatcaacgccgtcccggaagtgaagaaactggccaacgtcaagggtgagcaattctccaacatggccagcgagaacatgactggcgatgtggtactgaagctctcgcagcgcgtgaacgaactgctcgcccgcgacgacgtggacggcgtggtgatcacccacggcactgataccgtcgaagagtcggcgtactttctccacctgaccgtgaagtccgataagcccgtggtgtttgtcgccgcgatgcgcccggcgaccgccatcagcgccgacgggccgatgaatctgttggaagccgtgcgcgtggcgggtgacaagcaaagccgcggtcggggcgtaatggtcgtcctgaacgatcggatcggtagcgcgcggtacatcaccaagacgaacgcctccacgctggacaccttcaaggcgaacgaagaggggtacctgggggtgatcattggcaatcgtatctattaccagaaccgcatcgacaagctgcacaccacccgctcggtgttcgacgtgcgcggtctgactagcctgcccaaggtcgacatcctgtacggctaccaagacgacccggagtacctctacgacgcggcgatccagcatggcgtgaagggcatcgtctacgccggtatgggtgccggctcggtgtcggtccgcggcatcgcgggtatgcgcaaggccatggagaaaggcgtggtcgtgattcgctcgacccggactggcaatggcatcgtaccgcccgatgaagaactcccggggctcgtgagcgatagcctcaaccccgcgcacgcccggatcctgctgatgctggcgctcacgcggaccagcgaccccaaggtcattcaagagtacttccacacctac

SEQ ID NO: 9 - protein, 326 aa, Escherichia coli
LPNITILATGGTIAGGGDSATKSNYTAGKVGVENLVNAVPQLKDIANVKGEQVVNIGSQDMNDDVWLTLAKKINTDCDKTDGFVITHGTDTMEETAYFLDLTVKCDKPVVMVGAMRPSTSMSADGPFNLYNAVVTAADKASANRGVLVVMNDTVLDGRDVTKTNTTDVATFKSVNYGPLGYIHNGKIDYQRTPARKHTSDTPFDVSKLNELPKVGIVYNYANASDLPAKALVDAGYDGIVSAGVGNGNLYKTVFDTLATAAKNGTAVVRSSRVPTGATTQDAEVDDAKYGFVASGTLNPQKARVLLQLALTQTKDPQQIQQIFNQY

SEQ ID NO: 10 - DNA, 978 bp, Artificial Sequence
  Description of Artificial Sequence: Synthetic polynucleotide
ctccctaacattactattctggccactggcggtacgattgcaggcggcggtgactcagccaccaagtcgaattacaccgccggtaaggtcggtgtcgaaaacctcgtcaacgccgtgccgcagctgaaagatatcgccaacgtcaagggcgagcaagtggtgaacatcggctcccaagatatgaacgatgacgtgtggctgacgctggccaagaaaatcaacaccgattgcgacaagacggacgggtttgtcatcacccacggcaccgacactatggaagagactgcctacttcctcgacctcacggtgaagtgcgataaaccggtagtgatggtgggcgccatgcgcccgagcacctcgatgagcgcggacggcccgttcaatctgtacaacgccgtggtaaccgcagcggacaaggcgtccgcgaaccgcggtgtattggtagtgatgaacgatacggtgctcgatgggcgcgatgtgaccaagaccaataccactgatgtggccaccttcaagagcgtgaactatggcccgctgggctacatccataacggcaagatcgattaccagcgtactcccgcccggaagcacacctcggacacccccttcgacgtgtcgaaactgaacgaactgcccaaggtcggcatcgtctacaactacgccaatgcgagcgatctgcccgcgaaggccctggtggacgccggctacgacgggatcgtatcggcgggtgtgggcaatggtaacctgtacaagaccgtgtttgacaccctggcgacggcggcgaagaacggcaccgccgtggtccgcagcagccgcgtgcccactggggcgaccacccaagacgccgaggtcgacgacgcgaagtacggcttcgtagccagcggcaccctgaacccgcaaaaggcccgggtcctgctgcagctggcgctcacgcagacgaaggacccgcagcaaatccaacagatcttcaaccagtac

SEQ ID NO: 11 - DNA, 6 bp, Artificial Sequence
  Description of Artificial Sequence: Synthetic oligonucleotide
aggagg

SEQ ID NO: 12 - DNA, 6 bp, Unknown
  Description of Unknown: RBS2 sequence
ggagcg

SEQ ID NO: 13 - DNA, 6 bp, Unknown
  Description of Unknown: RBS34 sequence
ggagcg

SEQ ID NO: 14 - DNA, 6 bp, Unknown
  Description of Unknown: RBS41 sequence
aggagt

SEQ ID NO: 15 - DNA, 6 bp, Unknown
  Description of Unknown: RBS43 sequence
ggagtg

SEQ ID NO: 16 - DNA, 6 bp, Unknown
  Description of Unknown: RBS48 sequence
gagtaa

SEQ ID NO: 17 - DNA, 6 bp, Unknown
  Description of Unknown: RBS1 sequence
agagag

SEQ ID NO: 18 - DNA, 6 bp, Unknown
  Description of Unknown: RBS35 sequence
aaggca

SEQ ID NO: 19 - DNA, 6 bp, Unknown
  Description of Unknown: RBS49 sequence
ccgaac

SEQ ID NO: 20 - DNA, 1020 bp, Artificial Sequence
  Description of Artificial Sequence: Synthetic polynucleotide
atatgctcttcagccgcagacaaactccctaacatcgtaatcctcgcaactggtggtaccatcgcaggcagcgccgccaccggcacgcagaccactggctacaaggccggcgcgctgggcgtagacacgctgatcaacgccgtcccggaagtgaagaaactggccaacgtcaagggtgagcaattctccaacatggccagcgagaacatgactggcgatgtggtactgaagctctcgcagcgcgtgaacgaactgctcgcccgcgacgacgtggacggcgtggtgatcacccacggcactgataccgtcgaagagtcggcgtactttctccacctgaccgtgaagtccgataagcccgtggtgtttgtcgccgcgatgcgcccggcgaccgccatcagcgccgacgggccgatgaatctgttggaagccgtgcgcgtggcgggtgacaagcaaagccgcggtcggggcgtaatggtcgtcctgaacgatcggatcggtagcgcgcggtacatcaccaagacgaacgcctccacgctggacaccttcaaggcgaacgaagaggggtacctgggggtgatcattggcaatcgtatctattaccagaaccgcatcgacaagctgcacaccacccgctcggtgttcgacgtgcgcggtctgactagcctgcccaaggtcgacatcctgtacggctaccaagacgacccggagtacctctacgacgcggcgatccagcatggcgtgaagggcatcgtctacgccggtatgggtgccggctcggtgtcggtccgcggcatcgcgggtatgcgcaaggccatggagaaaggcgtggtcgtgattcgctcgacccggactggcaatggcatcgtaccgcccgatgaagaactcccggggctcgtgagcgatagcctcaaccccgcgcacgcccggatcctgctgatgctggcgctcacgcggaccagcgaccccaaggtcattcaagagtacttccacacctactgataatagttcagaagagcatat